European Patent Specification EP 3 816 184 B1, published April 26, 2023. Title: Anti-human interleukin 17A monoclonal antibody and application thereof. Applicant: JIANGSU QYUNS THERAPEUTICS CO., LTD. Application EP 18919093.7. The sequence listing filed with the application follows.

SEQUENCE LISTING (11 sequences)

SEQ ID NO: 1 - protein, 5 aa, Artificial Sequence
  artificially synthesized sequence
LFYMS

SEQ ID NO: 2 - protein, 15 aa, Artificial Sequence
  artificially synthesized sequence
TIHEVASSYYASWAK

SEQ ID NO: 3 - protein, 12 aa, Artificial Sequence
  artificially synthesized sequence
ETYSSRYPYPNI

SEQ ID NO: 4 - protein, 11 aa, Artificial Sequence
  artificially synthesized sequence
QASQNIGGSLA

SEQ ID NO: 5 - protein, 7 aa, Artificial Sequence
  artificially synthesized sequence
GASSLAS

SEQ ID NO: 6 - protein, 12 aa, Artificial Sequence
  artificially synthesized sequence
QSYNTISTYGLA

SEQ ID NO: 7 - protein, 120 aa, Artificial Sequence
  artificially synthesized sequence
EVQLQESGPGLVKPSETLSLTCTVSGIDLSLFYMSWIRQPPGKGLEWIGTIHEVASSYYASWAKGRVTISKDTSKNQFSLKLSSVTAADTAVYYCARETYSSRYPYPNIWGQGTLVTVSS

SEQ ID NO: 8 - protein, 110 aa, Artificial Sequence
  artificially synthesized sequence
DIQMTQSPSSVSASVGDRVTITCQASQNIGGSLAWYQQKPGKAPKLLIYGASSLASGVPSRFSGSGSGTDFTLTISSLQPEDFATYYCQSYNTISTYGLAFGGGTKVEIK

SEQ ID NO: 9 - protein, 155 aa, Homo sapiens
  artificially synthesized sequence
MTPGKTSLVSLLLLLSLEAIVKAGITIPRNPGCPNSEDKNFPRTVMVNLNIHNRNTNTNPKRSSDYYNRSTSPWNLHRNEDPERYPSVIWEAKCRHLGCINADGNVDYHMNSVPIQQEILVLRREPPHCPNSFRLEKILVSVGCTCVTPIVHHVA

SEQ ID NO: 10 - protein, 450 aa, Artificial Sequence
  artificially synthesized sequence
EVQLQESGPGLVKPSETLSLTCTVSGIDLSLFYMSWIRQPPGKGLEWIGTIHEVASSYYASWAKGRVTISKDTSKNQFSLKLSSVTAADTAVYYCARETYSSRYPYPNIWGQGTLVTVSSASTKGPSVFPLAPSSKSTSGGTAALGCLVKDYFPEPVTVSWNSGALTSGVHTFPAVLQSSGLYSLSSVVTVPSSSLGTQTYICNVNHKPSNTKVDKKVEPKSCDKTHTCPPCPAPELLGGPSVFLFPPKPKDTLMISRTPEVTCVVVDVSHEDPEVKFNWYVDGVEVHNAKTKPREEQYNSTYRVVSVLTVLHQDWLNGKEYKCKVSNKALPAPIEKTISKAKGQPREPQVYTLPPSRDELTKNQVSLTCLVKGFYPSDIAVEWESNGQPENNYKTTPPVLDSDGSFFLYSKLTVDKSRWQQGNVFSCSVMHEALHNHYTQKSLSLSPGK

SEQ ID NO: 11 - protein, 217 aa, Artificial Sequence
  artificially synthesized sequence
DIQMTQSPSSVSASVGDRVTITCQASQNIGGSLAWYQQKPGKAPKLLIYGASSLASGVPSRFSGSGSGTDFTLTISSLQPEDFATYYCQSYNTISTYGLAFGGGTKVEIKRTVAAPSVFIFPPSDEQLKSGTASVVCLLNNFYPREAKVQWKVDNALQSGNSQESVTEQDSKDSTYSLSSTLTLSKADYEKHKVYACEVTHQGLSSPVTKSFNRGEC